European Patent Specification EP 3 535 392 B1, published March 27, 2024. Title: Immunologically Discernible Cell Surface Variants for Use in Cell Therapy. Applicant: Universität Basel. The sequence listing filed with the application follows.

SEQUENCE LISTING (32 sequences)

SEQ ID NO: 1 - DNA, 20 bp, Mus musculus
gttttgtgagcttcaagtct

SEQ ID NO: 2 - DNA, 20 bp, Mus musculus
gtttgtgagcttcgagtctc

SEQ ID NO: 3 - DNA, 20 bp, Mus musculus
ggctaatacttcaatttgtt

SEQ ID NO: 4 - DNA, 20 bp, Mus musculus
ttggagtggaaaacagaaaa

SEQ ID NO: 5 - DNA, 20 bp, Mus musculus
aacaaaaaaccttgatttca

SEQ ID NO: 6 - DNA, 20 bp, Mus musculus
aaacaaaaaaccttgatttc

SEQ ID NO: 7 - DNA, 180 bp, Mus musculus
cgtcaccctctccaaccagccctatatcaaggtccttaccctagccaacttcaccaccaaggatgagggcgactacttttgtgagcttcgagtctcgggcgcgaatcccatgagctccaataaaagtatcagtgtgtatagaggtgagactggttcccagaaagataaaatgtccaggtt

SEQ ID NO: 8 - DNA, 180 bp, Mus musculus
cgtcaccctctccaaccagccctatatcaaggtccttaccctagccaacttcaccaccaaggatgagggcgactacttttgtgagcttcgagtctcaggcgcgaatcccatgagctccaataaaagtatcagtgtgtatagaggtgagactggttcccagaaagataaaatgtccaggtt

SEQ ID NO: 9 - DNA, 179 bp, Mus musculus
cgtcaccctctccaaccagccctatatcaaggtccttaccctagccaacttcaccaccaaggatgagggcgactacttttgtgagcttcgagtaagcggagcgaatcccatgagctccaataaaagtatcagtgtgtatagaggtgagactggttcccagaaagataaaatgtccaggt

SEQ ID NO: 10 - DNA, 2000 bp, Mus musculus
aaatggggacccacctgtcctaccagctggctgacctgtagctttccccaccacagaatccaagtcggaactcttggcaccatgaacccagccatcagcgtcgctctcctgctctcaggtactgggcaagggtcagggctggcattctaaggaatctggcttcctcccatcccgggaagtagcctctttgccatagtctcaggggcacaggtggttgggaggtgcgggggtggggagtggggaggagcctcaacctcaccagtggtggtctttgacatattagaaactccataatggatctaggaactcctcttgctgggtggtggtggttgtggtacacacctttaatctcagcactcaggaggcagagtcaggtggatctgttagtctgaagccagcctggtctacagagcaaattccaggacagccagagctattctcaagatagagaatccctttcttgaaaaaaccatttaaaaacaaaaacaaaagcaacacactcctcttgatctcctgttcttgaaacacattgttgggacccagaacttcagtagattgatggaagttggagtctgcaagtggtggaacatcccaccaatacctcaagggcgagtgcaaaccccacatccccccagctcaagtctacttttcctgcaggtgggaggccccgggtctgtgtctccccaaattcagagaaggcactgctgtgccagtcttgcaggtgtcccgagggcagaaggtgaccagcctgacagcctgcctggtgaaccaaaaccttcgcctggactgccgccatgagaataacaccaaggataactccatccagcatgagttcagcctgacccgagagaagaggaagcacgtgctctcaggcacccttgggatacccgagcacacgtaccgctcccgcgtcaccctctccaaccagccctatatcaaggtccttaccctagccaacttcaccaccaaggatgagggcgactacttttgtgagcttcgagtctcaggcgcgaatcccatgagctccaataaaagtatcagtgtgtatagaggtgagactggttcccagaaagataaaatgtccaggttagccaggctggggtagccaataaaaaaaaaaaaaaaaaaaaaaaaaaaaacaggcacctccattacccttcccctaactgctggtctcctgggaaactgctgctgtctatgtgagtggggcaagattaggggccagaaagggggagcttgtagtaaaagcacagttgaggaaactaaatgggaaaggcagtacagtggtgattcttgtggtgtggaggttctgttacagcatccggtggagccgctaagatgagaaagcgccagctagctgccttgaacagctgacacctgtctttgcccgcctgagtcctgatctcccctcctcccggcaccccttctctatccacagacaagctggtcaagtgtggcggcataagcctgctggttcagaacacatcctggatgctgctgctgctgctttccctctccctcctccaagccctggacttcatttctctgtgactggttgggcccaaggagaaacaggagccctcgaggtccttcctctgcagaggtcttgcttctcccggtcagctgactccctccccaagtccttcaaatatctcagaacatggggagaaacggggaccttgtccctcctaaggaaccccagtgctgcatgccatcatcccccccaccctcgcccccacccccgccacttctccctccatgcataccactagctgtcattttgtactctgtatttattccagggctgcttctgattatttagtttgttctttccctggagacctgttagaacataagggcgtatggtgggtaggggaggcaggatatcagtccctggggcgagttcctccctgccaaccaagccagatgcctgaaagagatatggatgagggaagttggactgtgcctgtacctggtacagtcatactctgttgaaagaa

SEQ ID NO: 11 - DNA, 3679 bp, Mus musculus
accccatcaaaatcctatttgagtgtacggttcggagaacctcatttatccggtaaatgtcttttactctgctctcagggagctgaggcaggacatcctgagatacattgggagaggagatacagtttcaataaaataataggttgggtggaggtacatgcctataatgccaccactcaggaaatggtggcagcttcgtgagtttgaggccaacccaagaaacatagtgaaaccctgtcagtaaataagtaagcaagtatttgagtatctactatatgctagggctgacctggacattaggggtcatcttctgaacaaactagtgcttgagggaggtatttggggtttttgtttgtttaatggatctgaatgagttccagagactggctacacagcgatatgactgagcttaacacccctaaagcatacagtcagaccaattagacaataaaaggtatgtatagcttaccaaataaaaaaattgtattttcaagagagtgtctgtctgtgtagccctggctgttcttgaactcactctgtagaccaggctggcctggaaatccatctgcctgcctctgcctctctgcctctctgcctctctgcctctctctctgcctctctctgcctctctctgcccctctctgcccctctctgcccctctctgcccctctctgccgccctctgccttctgccctctgccctctggcctctggcctctgccctctgccctctggcctctggcctctgcctctgcctcttgagtgctggaatcaaaggtgtgagctctgtaggtcttaagttccagaagaaagtaatgaagtcacccagcagggaggtgctcagggacagcacagacacacacccaggacataggctcccacttccttggctttctctgagtggcaaaggaccttaggcagtgtcactccctaagagaaggggataaagagaggggctgaggtattcatcatgtgctccgtggatctcaagccctcaaggtaaatggggacccacctgtcctaccagctggctgacctgtagctttccccaccacagaatccaagtcggaactcttggcaccatgaacccagccatcagcgtcgctctcctgctctcaggtactgggcaagggtcagggctggcattctaaggaatctggcttcctcccatcccgggaagtagcctctttgccatagtctcaggggcacaggtggttgggaggtgcgggggtggggagtggggaggagcctcaacctcaccagtggtggtctttgacatattagaaactccataatggatctaggaactcctcttgctgggtggtggtggttgtggtacacacctttaatctcagcactcaggaggcagagtcaggtggatctgttagtctgaagccagcctggtctacagagcaaattccaggacagccagagctattctcaagatagagaatccctttcttgaaaaaaccatttaaaaacaaaaacaaaagcaacacactcctcttgatctcctgttcttgaaacacattgttgggacccagaacttcagtagattgatggaagttggagtctgcaagtggtggaacatcccaccaatacctcaagggcgagtgcaaaccccacatccccccagctcaagtctacttttcctgcaggtgggaggccccgggtctgtgtctccccaaattcagagaaggcactgctgtgccagtcttgcaggtgtcccgagggcagaaggtgaccagcctgacagcctgcctggtgaaccaaaaccttcgcctggactgccgccatgagaataacaccaaggataactccatccagcatgagttcagcctgacccgagagaagaggaagcacgtgctctcaggcacccttgggatacccgagcacacgtaccgctcccgcgtcaccctctccaaccagccctatatcaaggtccttaccctagccaacttcaccaccaaggatgagggcgactacttttgtgagcttcgagtctcaggcgcgaatcccatgagctccaataaaagtatcagtgtgtatagaggtgagactggttcccagaaagataaaatgtccaggttagccaggctggggtagccaataaaaaaaaaaaaaaaaaaaaaaaaaaaaacaggcacctccattacccttcccctaactgctggtctcctgggaaactgctgctgtctatgtgagtggggcaagattaggggccagaaagggggagcttgtagtaaaagcacagttgaggaaactaaatgggaaaggcagtacagtggtgattcttgtggtgtggaggttctgttacagcatccggtggagccgctaagatgagaaagcgccagctagctgccttgaacagctgacacctgtctttgcccgcctgagtcctgatctcccctcctcccggcaccccttctctatccacagacaagctggtcaagtgtggcggcataagcctgctggttcagaacacatcctggatgctgctgctgctgctttccctctccctcctccaagccctggacttcatttctctgtgactggttgggcccaaggagaaacaggagccctcgaggtccttcctctgcagaggtcttgcttctcccggtcagctgactccctccccaagtccttcaaatatctcagaacatggggagaaacggggaccttgtccctcctaaggaaccccagtgctgcatgccatcatcccccccaccctcgcccccacccccgccacttctccctccatgcataccactagctgtcattttgtactctgtatttattccagggctgcttctgattatttagtttgttctttccctggagacctgttagaacataagggcgtatggtgggtaggggaggcaggatatcagtccctggggcgagttcctccctgccaaccaagccagatgcctgaaagagatatggatgagggaagttggactgtgcctgtacctggtacagtcatactctgttgaaagaatcatcggggaggggggggggggctcaagatgggagagctctgctgagcctttgtggaccatccaatgaggatgagggcttagattctaccaggtcattctcagccaccacacacaagcgctctgccatcactgaagaagccccctagggctcttgggccagggcacactcagtaaagatgcaggttcagtcagggaatgatggggaaaggggtaggaggtgggggagggatcaccccctcctctaaaacacgagcctgctgtctccaaaggcctctgcctgtagtgagggtggcagaagaagacaaggagccagaactctgactccaggatctaagtccgtgcaggaaggggatcctagaaccatccggttggacccagcttaccaagggagagcctttattcttctttcccttgcccctctgtgccagcccctcttgctgtccctgatcccccagacagcgagagtcttgcaacctgcctcttccaagacctcctaatctcaggggcaggcggtggagtgagatccggcgtgcacactttttggaagatagctttcccaaggatcctctcccccactggcagctctgcctgtcccatcaccatgtataataccaccactgctacagcatctcaccgaggaaagaaaactgcacaataaaaccaagcctctggagtgtg

SEQ ID NO: 12 - DNA, 960 bp, Mus musculus
cacattgttgggacccagaacttcagtagattgatggaagttggagtctgcaagtggtggaacatcccaccaatacctcaagggcgagtgcaaaccccacatccccccagctcaagtctacttttcctgcaggtgggaggccccgggtctgtgtctccccaaattcagagaaggcactgctgtgccagtcttgcaggtgtcccgagggcagaaggtgaccagcctgacagcctgcctggtgaaccaaaaccttcgcctgactgccgccatgagaataacaccaaggataactccatccagcatgagttcagcctgacccgagagaagaggaagcacgtgctctcaggcacccttgggatacccgagcacacgtaccgctcccgcgtcaccctctccaaccagccctatatcaaggtccttaccctagccaacttcaccaccaaggatgagggcgactacttttgtgagcttcgagtctcaggcgcgaatcccatgagctccaataaaagtatcagtgtgtatagaggtgagactggttcccagaaagataaaatgtccaggttagccaggctggggtagccaataaaaaaaaaaaaaaaaaaaaaaaaaaaaacaggcacctccattacccttcccctaactgctggtctcctgggaaactgctgctgtctatgtgagtggggcaagattaggggccagaaagggggagcttgtagtaaaagcacagttgaggaaactaaatgggaaaggcagtacagtggtgattcttgtggtgtggaggttctgttacagcatccggtggagccgctaagatgagaaagcgccagctagctgccttgaacagctgacacctgtctttgcccgcctgagtcctgatctcccctcctcccggcaccccttctctatccacagacaagctggtcaagtgtggcggcataagcctgctggttcagaacacat

SEQ ID NO: 13 - DNA, 160 bp, Mus musculus
cgtcaccctctccaaccagccctatatcaaggtccttaccctagccaacttcaccaccaaggatgagggcgactacttttgtgagcttcgagtctcaggcgcgaatcccatgagctccaataaaagtatcagtgtgtatagaggtgagactggttcccag

SEQ ID NO: 14 - DNA, 120 bp, Mus musculus
agtttgtctctatacacactgatacttttattggagctcatgggattcgcgcccgagacttgaagctcacaaaagtagtcgccctcatccttggtggtgaagttggctagggtaaggacc

SEQ ID NO: 15 - DNA, 180 bp, Mus musculus
accagcaggcttatgccgccacacttgaccagtttgtctctatacacactgatacttttattggagctcatgggattcgcgcccgagacttgaagctcacaaaagtagtcgccctcatccttggtggtgaagttggctagggtaaggaccttgatatagggctggttggagagggtgacg

SEQ ID NO: 16 - DNA, 180 bp, Mus musculus
gtttcctccacagggactgacaagttttcgctacatgactgcacaccaaaagaaaaggctaatacttcaatttgtttagagtggaaaacagaaaaccttgatttcagaaaatgcaacagtgacaatatttcatatgtactccactgtgagccaggtacgatgctgggcagagaagttcta

SEQ ID NO: 17 - DNA, 1000 bp, Mus musculus
caaatgggaaaaatcagccgtttatcttgatgtttccttgagttgcatttataaaagcagcacacatttctactgaaatctgtggtacgaagaaaatatgttatcttccctaatgaatggcaaatatctgagttgataaacaaactgccagcaagtggtgtctacacatatagatatatcaaaacactaataatgtgcacatatttgtataattgtgcatcagctgaaatggagataaattaaaaattaggaatgtgactagatcatgaagaagcatcagaccttgggagagcttagatgtcccctagcgaaatctcctgcttgcaagactgtactccatgagtcttatttcagagttgagagggttcacatctccacaccaggaaccatcacctaagagcacctctccgtttcctccacagggactgacaagttttcgctacatgactgcacaccaaaagaaaaggctaatacttcaatttgtttagagtggaaaacagaaaaccttgatttcagaaaatgcaacagtgacaatatttcatatgtactccactgtgagccaggtacgatgctgggcagagaagttctattatcagaaattattccagacgtggcttaaatgttctttctgtagccttgtcctcctcacccaccctcagtgatccgccataaattagaataaaataaccctagtatctctggcactgaaacaaattcacaacgtagataaatgaaaagagcaacccatggatgataaatattatgaaaaattaattaaaagaattttcttgagtactgttatataccagacattgttgaaagggtgatgagatgcaggcattataaaagaaagatggtatccatagtctgtagaaaggaagcatagtattatccacaccggaggttgctttctcagactttcatacatgaaaatcattggaaagttcaagaatctgcaggtagcaaggaaaacaagtgcttctaggagggaacatgggtt

SEQ ID NO: 18 - DNA, 1995 bp, Mus musculus
atggtttacagagcaagtttcaagacagcccaggatacacagagaaaccctgtctcaaaacaaacaaaacaaaacaaaaagcaaaaaacacaaaactaaaacaacataacaacaaaccatcaaaaagcagttcctatggattagaaacagcctattttgtattttgtgaaataattatacataagattgctgttttttcatttttttctttcttctttttggtatttctttttaaattcaaaatgttctcattagagaaaagaatgtagttaaacatctaatgttttctggaaaaaaaaatcaaagggggaattctagttatgttaataccaaagttgtgatcacagcacgtggaaggcaggagtaccttatgtgttcaaagccagtctatgctgtatcttgaattctgtggcagccttcacagtgtgagattacaccttgtttccaaaaccccaaacagatcaacaacaagcgtgaaaacagcaaagaaattgtttttcaaatgggaaaaatcagccgtttatcttgatgtttccttgagttgcatttataaaagcagcacacatttctactgaaatctgtggtacgaagaaaatatgttatcttccctaatgaatggcaaatatctgagttgataaacaaactgccagcaagtggtgtctacacatatagatatatcaaaacactaataatgtgcacatatttgtataattgtgcatcagctgaaatggagataaattaaaaattaggaatgtgactagatcatgaagaagcatcagaccttgggagagcttagatgtcccctagcgaaatctcctgcttgcaagactgtactccatgagtcttatttcagagttgagagggttcacatctccacaccaggaaccatcacctaagagcacctctccgtttcctccacagggactgacaagttttcgctacatgactgcacaccaaaagaaaaggctaatacttcaatttgtttagagtggaaaacagaaaaccttgatttcagaaaatgcaacagtgacaatatttcatatgtactccactgtgagccaggtacgatgctgggcagagaagttctattatcagaaattattccagacgtggcttaaatgttctttctgtagccttgtcctcctcacccaccctcagtgatccgccataaattagaataaaataaccctagtatctctggcactgaaacaaattcacaacgtagataaatgaaaagagcaacccatggatgataaatattatgaaaaattaattaaaagaattttcttgagtactgttatataccagacattgttgaaagggtgatgagatgcaggcattataaaagaaagatggtatccatagtctgtagaaaggaagcatagtattatccacaccggaggttgctttctcagactttcatacatgaaaatcattggaaagttcaagaatctgcaggtagcaaggaaaacaagtgcttctaggagggaacatgggtttctctagaggttggatcttttaaaacatatatttgaattcagtgaggtggactctttctcctctaggcatacagctatgtgccaggacacacttgacaagacagagggaggtacatacacccagaggcggaagaggaaatttcactctgattgtaaacattgtgctaacaggaaattgctgggctaagatacaaataggatgttcacagctggaacaaatatatgttgagttaacatttttttaaaaaattttaaataagtcacaatactgatttctcaacaaaattgagtatagcaatgttatctgcaggatcttggtttattatttcaccattttcagagacttgaccttaacatgaagtcttaaacacatggtgccataaaagaagcccatttactatgtggcatttcatatactcatgtgcaatacttacttctttcagaaaataatacaaaatgcattagaagaaatacattcatacctgaaagatgtcag

SEQ ID NO: 19 - DNA, 4000 bp, Mus musculus
ttaattcaccaagtattattgaattgttgataacagacagatatatcataaacccgagttaatgataatgaacaaaatagactagttatggttctcatggacttttcaatttagttggaaagatagataccaaaccaataattatcatagtataaactgggatcttttataggagaaaggatttcaaaataatgatgtaggggtacatgatacagttcttctatttttcatattcctggagatactgtgctacaacctacaatctgctttggtgatattttggtatattacctctgctatatgctaattattcttttacttctgcttgctgagtactgaatttgaaacccaaaatacacttatttcatcagatcattctctgtacaaaagaatatgttaagacatttgtatccaatgtagtatcattcattctcgatgatgattgtactaatttcctttttttttttttccagctgccatgtttgggaacattactgtgaattacacctatgaatctagtaatcagacttttaaggcagacctcaaagatgtccaaaatgctaagtgtggaaatgaggattgtgaaaacgtgttaaataatctagaagaatgctcacagataaaaaacatcagtgtgtctaatgactcatgtgctccagctacaactatagatttatatgtaccaccaggtgaatgtcaatttctctctatctgggtatttagagcaacagaaggatttcatgtatgtgttcctgtgcttcttcaagctaatgtggtcagaaaaaagaaccgagggaaagcaagtgagctttgataagagtgtgtttcctgctgagaaccccggagagcagagagaaatacacacttattccttaggaccaccacctggctctcttatttcttttataaagagattcccagctgggaagtggtgtccctcaccttcaatctcagcacttcagaggcagaggcaggcagatctcagggttccaaggcagccatggtttacagagcaagtttcaagacagcccaggatacacagagaaaccctgtctcaaaacaaacaaaacaaaacaaaaagcaaaaaacacaaaactaaaacaacataacaacaaaccatcaaaaagcagttcctatggattagaaacagcctattttgtattttgtgaaataattatacataagattgctgttttttcatttttttctttcttctttttggtatttctttttaaattcaaaatgttctcattagagaaaagaatgtagttaaacatctaatgttttctggaaaaaaaaatcaaagggggaattctagttatgttaataccaaagttgtgatcacagcacgtggaaggcaggagtaccttatgtgttcaaagccagtctatgctgtatcttgaattctgtggcagccttcacagtgtgagattacaccttgtttccaaaaccccaaacagatcaacaacaagcgtgaaaacagcaaagaaattgtttttcaaatgggaaaaatcagccgtttatcttgatgtttccttgagttgcatttataaaagcagcacacatttctactgaaatctgtggtacgaagaaaatatgttatcttccctaatgaatggcaaatatctgagttgataaacaaactgccagcaagtggtgtctacacatatagatatatcaaaacactaataatgtgcacatatttgtataattgtgcatcagctgaaatggagataaattaaaaattaggaatgtgactagatcatgaagaagcatcagaccttgggagagcttagatgtcccctagcgaaatctcctgcttgcaagactgtactccatgagtcttatttcagagttgagagggttcacatctccacaccaggaaccatcacctaagagcacctctccgtttcctccacagggactgacaagttttcgctacatgactgcacaccaaaagaaaaggctaatacttcaatttgtttagagtggaaaacagaaaaccttgatttcagaaaatgcaacagtgacaatatttcatatgtactccactgtgagccaggtacgatgctgggcagagaagttctattatcagaaattattccagacgtggcttaaatgttctttctgtagccttgtcctcctcacccaccctcagtgatccgccataaattagaataaaataaccctagtatctctggcactgaaacaaattcacaacgtagataaatgaaaagagcaacccatggatgataaatattatgaaaaattaattaaaagaattttcttgagtactgttatataccagacattgttgaaagggtgatgagatgcaggcattataaaagaaagatggtatccatagtctgtagaaaggaagcatagtattatccacaccggaggttgctttctcagactttcatacatgaaaatcattggaaagttcaagaatctgcaggtagcaaggaaaacaagtgcttctaggagggaacatgggtttctctagaggttggatcttttaaaacatatatttgaattcagtgaggtggactctttctcctctaggcatacagctatgtgccaggacacacttgacaagacagagggaggtacatacacccagaggcggaagaggaaatttcactctgattgtaaacattgtgctaacaggaaattgctgggctaagatacaaataggatgttcacagctggaacaaatatatgttgagttaacatttttttaaaaaattttaaataagtcacaatactgatttctcaacaaaattgagtatagcaatgttatctgcaggatcttggtttattatttcaccattttcagagacttgaccttaacatgaagtcttaaacacatggtgccataaaagaagcccatttactatgtggcatttcatatactcatgtgcaatacttacttctttcagaaaataatacaaaatgcattagaagaaatacattcatacctgaaagatgtcagttggacaaccttcgtgcccaaacaaattacacatgtgtagcagaaatcttatatcgcggtgtaaaactcgtcaaaaatgttataaatgtgcagacagatttggggagtaagtatatcgtttatgtttataaaataaataaaatttctttttcttttatgggtttacttttatttttggagagtcatagaaaataatggtatagaattacagaaagcatatcagtgaagaaaaaagtttaaatgcactttaaggtcaattttaaaaactaggttatacaaacctaactaaagttctttttctgttgttcaaattgtgtctgccgtaagtctggtagaaacacttgaaatggtttacatagattattcccattttattcattttctcctcccttctttttataacaccatttgttctgtattctaacacttctttcacaattatgctctgcttctaatagaaataaaataagcaaagaaactaataaaactcaagcaaatctacatgtttaaacataaaatacggagtatagttatcaaattttggcaatagaattaataaccggataaaccttattaaatagaaaggggttctacttgggaagtcagatgtgaaattttcaaattaaatgtaacatttgatggtaaatgctaattttttaaaatggtgattaatgaataatcaaccataaagaagacaaaagatgtcattgctcacaagcagtaaagacatttttagaaggaagagaagagaagcagtaggaaaggaggaagggagagatagatgatagatagataatagatagatagatagatagatagatagatagatagagacagacagacagacagaaagaaagagagagacagaaacagagagacacaaaaaaagaggaaagagaagactgggagaaagggaaagtaagggatggagaaaaaagggagagagataaaaagaagacaaaaacataaatgaaagcaaggaatgatgatatatatctgttatgt

SEQ ID NO: 20 - DNA, 57 bp, Mus musculus
ttttgtgagcttcgagtctcggtcgcgaatcccatgagctccaataaaagtatcagt

SEQ ID NO: 21 - DNA, 57 bp, Mus musculus
ttttgtgagcttcaagtctcggtcgcgaatcccatgagctccaataaaagtatcagt

SEQ ID NO: 22 - DNA, 63 bp, Mus musculus
aaaaggctaatacttcaatttgtttggagtggaaaacaaaaaaccttgatttcagaaaatgca

SEQ ID NO: 23 - DNA, 63 bp, Mus musculus
aaaaggctaatacttcaatttgtttagagtggaaaacagaaaaccttgatttcagaaaatgca

SEQ ID NO: 24 - DNA, 48 bp, Mus musculus
ggctaatacttcaatttgtttggagtggaaaacagaaaaccttgattt

SEQ ID NO: 25 - DNA, 48 bp, Mus musculus
ggctaatacttcaatttgtttggagtggaaaacaaaaaaccttgattt

SEQ ID NO: 26 - DNA, 64 bp, Mus musculus
ggctaatacttcaatttgtttggagtggaaaacaaaaaaccttgatttcagaaaatgcaacagt

SEQ ID NO: 27 - DNA, 64 bp, Mus musculus
ggctaatacttcaatttgtttagagtggaaaacagaaaaccttgatttcagaaaatgcaacagt

SEQ ID NO: 28 - DNA, 63 bp, Mus musculus
gcctcaatggacaagagctcttgctgcatcgtagccaccagtactcagggcagtgtgctcccg

SEQ ID NO: 29 - DNA, 63 bp, Mus musculus
gcctcaatggactagatatcttgctgcatcgtagccaccagtactcagggcagtgtgctcccg

SEQ ID NO: 30 - DNA, 63 bp, Mus musculus
gcctcaatggacaaaagagctcttgctgcatcgtagccaccagtactcagggcagtgtgctcc

SEQ ID NO: 31 - DNA, 34 bp, Mus musculus
gcctcaatggacaagagctcttgctgcatcgtag

SEQ ID NO: 32 - DNA, 34 bp, Mus musculus
gcctcaatggactagatatcttgctgcatcgtag